European Patent Specification EP 3 732 185 B1, published February 26, 2025. Title: CONJUGATES AND PREPARATION AND USE THEREOF. Applicant: Suzhou Ribo Life Science Co.,Ltd. The sequence listing filed with the application follows.

SEQUENCE LISTING (251 sequences)

SEQ ID NO: 1 - RNA, 19 nt, Artificial sequence
  sense sequence for siHBa1
ccuugaggcauacuucaaa

SEQ ID NO: 2 - RNA, 21 nt, Artificial sequence
  Antisense sequence for siHBa1
uuugaaguaugccucaagguu

SEQ ID NO: 3 - RNA, 21 nt, Artificial sequence
  Sense sequence for siHBa2
gaccuugaggcauacuucaaa

SEQ ID NO: 4 - RNA, 23 nt, Artificial sequence
  Antisense sequence for siHBa2
uuugaaguaugccucaaggucgg

SEQ ID NO: 5 - RNA, 19 nt, Artificial sequence
  Sense sequence for siHBa1M1
ccuugaggcauacuucaaa

SEQ ID NO: 6 - RNA, 21 nt, Artificial sequence
  Antisense sequence for siHBa1M1
uuugaaguaugccucaagguu

SEQ ID NO: 7 - RNA, 19 nt, Artificial sequence
  Sense sequence for siHBa1M2
ccuugaggcauacuucaaa

SEQ ID NO: 8 - RNA, 21 nt, Artificial sequence
  Antisense sequence for siHBa1M2
uuugaaguaugccucaagguu

SEQ ID NO: 9 - RNA, 21 nt, Artificial sequence
  Sense sequence for siHBa2M1
gaccuugaggcauacuucaaa

SEQ ID NO: 10 - RNA, 23 nt, Artificial sequence
  Antisense sequence for siHBa2M1
uuugaaguaugccucaaggucgg

SEQ ID NO: 11 - RNA, 21 nt, Artificial sequence
  Sense sequence for siHBa2M2
gaccuugaggcauacuucaaa

SEQ ID NO: 12 - RNA, 23 nt, Artificial sequence
  Antisense sequence for siHBa2M2
uuugaaguaugccucaaggucgg

SEQ ID NO: 13 - RNA, 19 nt, Artificial sequence
  Sense sequence for siHBa1M1S
ccuugaggcauacuucaaa

SEQ ID NO: 14 - RNA, 21 nt, Artificial sequence
  Antisense sequence for siHBa1M1S
uuugaaguaugccucaagguu

SEQ ID NO: 15 - RNA, 19 nt, Artificial sequence
  Sense sequence for siHBa1M2S
ccuugaggcauacuucaaa

SEQ ID NO: 16 - RNA, 21 nt, Artificial sequence
  Antisense sequence for siHBa1M2S
uuugaaguaugccucaagguu

SEQ ID NO: 17 - RNA, 21 nt, Artificial sequence
  Sense sequence for siHBa2M1S
gaccuugaggcauacuucaaa

SEQ ID NO: 18 - RNA, 23 nt, Artificial sequence
  Antisense sequence for siHBa2M1S
uuugaaguaugccucaaggucgg

SEQ ID NO: 19 - RNA, 21 nt, Artificial sequence
  Sense sequence for siHBa2M2S
gaccuugaggcauacuucaaa

SEQ ID NO: 20 - RNA, 23 nt, Artificial sequence
  Antisense sequence for siHBa2M2S
uuugaaguaugccucaaggucgg

SEQ ID NO: 21 - RNA, 21 nt, Artificial sequence
  Antisense sequence for siHBa1M1P1
uuugaaguaugccucaagguu

SEQ ID NO: 22 - RNA, 21 nt, Artificial sequence
  Antisense sequence for siHBa1M2P1
uuugaaguaugccucaagguu

SEQ ID NO: 23 - RNA, 23 nt, Artificial sequence
  Antisense sequence for siHBa2M1P1
uuugaaguaugccucaaggucgg

SEQ ID NO: 24 - RNA, 23 nt, Artificial sequence
  Antisense sequence for siHBa2M2P1
uuugaaguaugccucaaggucgg

SEQ ID NO: 25 - RNA, 21 nt, Artificial sequence
  Antisense sequence for siHBa1M1SP1
uuugaaguaugccucaagguu

SEQ ID NO: 26 - RNA, 21 nt, Artificial sequence
  Antisense sequence for siHBa1M2SP1
uuugaaguaugccucaagguu

SEQ ID NO: 27 - RNA, 23 nt, Artificial sequence
  Antisense sequence for siHBa2M1SP1
uuugaaguaugccucaaggucgg

SEQ ID NO: 28 - RNA, 23 nt, Artificial sequence
  Antisense sequence for siHBa2M2SP1
uuugaaguaugccucaaggucgg

SEQ ID NO: 29 - RNA, 19 nt, Artificial sequence
  Sense sequence for siHBb1
ugcuaugccucaucuucua

SEQ ID NO: 30 - RNA, 21 nt, Artificial sequence
  Antisense sequence for siHBb1
uagaagaugaggcauagcagc

SEQ ID NO: 31 - RNA, 21 nt, Artificial sequence
  Antisense sequence for siHBb2
uagaagaugaggcauagcauu

SEQ ID NO: 32 - RNA, 19 nt, Artificial sequence
  Sense sequence for siHBb1M1
ugcuaugccucaucuucua

SEQ ID NO: 33 - RNA, 21 nt, Artificial sequence
  Antisense sequence for siHBb1M1
uagaagaugaggcauagcagc

SEQ ID NO: 34 - RNA, 21 nt, Artificial sequence
  Antisense sequence for siHBb2M1
uagaagaugaggcauagcauu

SEQ ID NO: 35 - RNA, 19 nt, Artificial sequence
  Sense sequence for siHBb1M2
ugcuaugccucaucuucua

SEQ ID NO: 36 - RNA, 21 nt, Artificial sequence
  Antisense sequence for siHBb1M2
uagaagaugaggcauagcagc

SEQ ID NO: 37 - RNA, 21 nt, Artificial sequence
  Antisense sequence for siHBb2M2
uagaagaugaggcauagcauu

SEQ ID NO: 38 - RNA, 19 nt, Artificial sequence
  Sense sequence for siHBb1M1S
ugcuaugccucaucuucua

SEQ ID NO: 39 - RNA, 21 nt, Artificial sequence
  Antisense sequence for siHBb1M1S
uagaagaugaggcauagcagc

SEQ ID NO: 40 - RNA, 21 nt, Artificial sequence
  Antisense sequence for siHBb2M1S
uagaagaugaggcauagcauu

SEQ ID NO: 41 - RNA, 19 nt, Artificial sequence
  Sense sequence for siHBb1M2S
ugcuaugccucaucuucua

SEQ ID NO: 42 - RNA, 21 nt, Artificial sequence
  Antisense sequence for siHBb1M2S
uagaagaugaggcauagcagc

SEQ ID NO: 43 - RNA, 21 nt, Artificial sequence
  Antisense sequence for siHBb2M2S
uagaagaugaggcauagcauu

SEQ ID NO: 44 - RNA, 21 nt, Artificial sequence
  Antisense sequence for siHBb1M1P1
uagaagaugaggcauagcagc

SEQ ID NO: 45 - RNA, 21 nt, Artificial sequence
  Antisense sequence for siHBb2M1P1
uagaagaugaggcauagcauu

SEQ ID NO: 46 - RNA, 21 nt, Artificial sequence
  Antisense sequence for siHBb1M2P1
uagaagaugaggcauagcagc

SEQ ID NO: 47 - RNA, 21 nt, Artificial sequence
  Antisense sequence for siHBb2M2P1
uagaagaugaggcauagcauu

SEQ ID NO: 48 - RNA, 21 nt, Artificial sequence
  Antisense sequence for siHBb1M1SP1
uagaagaugaggcauagcagc

SEQ ID NO: 49 - RNA, 21 nt, Artificial sequence
  Antisense sequence for siHBb2M1SP1
uagaagaugaggcauagcauu

SEQ ID NO: 50 - RNA, 21 nt, Artificial sequence
  Antisense sequence for siHBb1M2SP1
uagaagaugaggcauagcagc

SEQ ID NO: 51 - RNA, 21 nt, Artificial sequence
  Antisense sequence for siHBb2M2SP1
uagaagaugaggcauagcauu

SEQ ID NO: 52 - RNA, 19 nt, Artificial sequence
  Sense sequence for siHBc1
ucugugccuucucaucuga

SEQ ID NO: 53 - RNA, 21 nt, Artificial sequence
  Antisense sequence for siHBc1
ucagaugagaaggcacagacg

SEQ ID NO: 54 - RNA, 19 nt, Artificial sequence
  Sense sequence for siHBc1M1
ucugugccuucucaucuga

SEQ ID NO: 55 - RNA, 21 nt, Artificial sequence
  Antisense sequence for siHBc1M1
ucagaugagaaggcacagacg

SEQ ID NO: 56 - RNA, 19 nt, Artificial sequence
  Sense sequence for siHBc1M2
ucugugccuucucaucuga

SEQ ID NO: 57 - RNA, 21 nt, Artificial sequence
  Antisense sequence for siHBc1M2
ucagaugagaaggcacagacg

SEQ ID NO: 58 - RNA, 19 nt, Artificial sequence
  Sense sequence for siHBc1M1S
ucugugccuucucaucuga

SEQ ID NO: 59 - RNA, 21 nt, Artificial sequence
  Antisense sequence for siHBc1M1S
ucagaugagaaggcacagacg

SEQ ID NO: 60 - RNA, 19 nt, Artificial sequence
  Sense sequence for siHBc1M2S
ucugugccuucucaucuga

SEQ ID NO: 61 - RNA, 21 nt, Artificial sequence
  Antisense sequence for siHBc1M2S
ucagaugagaaggcacagacg

SEQ ID NO: 62 - RNA, 21 nt, Artificial sequence
  Antisense sequence for siHBc1M1P1
ucagaugagaaggcacagacg

SEQ ID NO: 63 - RNA, 21 nt, Artificial sequence
  Antisense sequence for siHBc1M2P1
ucagaugagaaggcacagacg

SEQ ID NO: 64 - RNA, 21 nt, Artificial sequence
  Antisense sequence for siHBc1M1SP1
ucagaugagaaggcacagacg

SEQ ID NO: 65 - RNA, 21 nt, Artificial sequence
  Antisense sequence for siHBc1M2SP1
ucagaugagaaggcacagacg

SEQ ID NO: 66 - RNA, 19 nt, Artificial sequence
  Sense sequence for siHBd1
cgugugcacuucgcuucaa

SEQ ID NO: 67 - RNA, 21 nt, Artificial sequence
  Antisense sequence for siHBd1
uugaagcgaagugcacacggu

SEQ ID NO: 68 - RNA, 19 nt, Artificial sequence
  Sense sequence for siHBd1M1
cgugugcacuucgcuucaa

SEQ ID NO: 69 - RNA, 21 nt, Artificial sequence
  Antisense sequence for siHBd1M1
uugaagcgaagugcacacggu

SEQ ID NO: 70 - RNA, 19 nt, Artificial sequence
  Sense sequence for siHBd1M2
cgugugcacuucgcuucaa

SEQ ID NO: 71 - RNA, 21 nt, Artificial sequence
  Antisense sequence for siHBd1M2
uugaagcgaagugcacacggu

SEQ ID NO: 72 - RNA, 19 nt, Artificial sequence
  Sense sequence for siHBd1M1S
cgugugcacuucgcuucaa

SEQ ID NO: 73 - RNA, 21 nt, Artificial sequence
  Antisense sequence for siHBd1M1S
uugaagcgaagugcacacggu

SEQ ID NO: 74 - RNA, 19 nt, Artificial sequence
  Sense sequence for siHBd1M2S
cgugugcacuucgcuucaa

SEQ ID NO: 75 - RNA, 21 nt, Artificial sequence
  Antisense sequence for siHBd1M2S
uugaagcgaagugcacacggu

SEQ ID NO: 76 - RNA, 21 nt, Artificial sequence
  Antisense sequence for siHBd1M1P1
uugaagcgaagugcacacggu

SEQ ID NO: 77 - RNA, 21 nt, Artificial sequence
  Antisense sequence for siHBd1M2P1
uugaagcgaagugcacacggu

SEQ ID NO: 78 - RNA, 21 nt, Artificial sequence
  Antisense sequence for siHBd1M1SP1
uugaagcgaagugcacacggu

SEQ ID NO: 79 - RNA, 21 nt, Artificial sequence
  Antisense sequence for siHBd1M2SP1
uugaagcgaagugcacacggu

SEQ ID NO: 80 - RNA, 19 nt, Artificial sequence
  Sense sequence for siAN1
ccaagagcaccaagaacua

SEQ ID NO: 81 - RNA, 21 nt, Artificial sequence
  Antisense sequence for siAN1
uaguucuuggugcucuuggcu

SEQ ID NO: 82 - RNA, 21 nt, Artificial sequence
  Sense sequence for siAN2
agccaagagcaccaagaacua

SEQ ID NO: 83 - RNA, 23 nt, Artificial sequence
  Antisense sequence for siAN2
uaguucuuggugcucuuggcuug

SEQ ID NO: 84 - RNA, 19 nt, Artificial sequence
  Sense sequence for siAN1M1
ccaagagcaccaagaacua

SEQ ID NO: 85 - RNA, 21 nt, Artificial sequence
  Antisense sequence for siAN1M1
uaguucuuggugcucuuggcu

SEQ ID NO: 86 - RNA, 21 nt, Artificial sequence
  Sense sequence for siAN2M1
agccaagagcaccaagaacua

SEQ ID NO: 87 - RNA, 23 nt, Artificial sequence
  Antisense sequence for siAN2M1
uaguucuuggugcucuuggcuug

SEQ ID NO: 88 - RNA, 21 nt, Artificial sequence
  Antisense sequence for siAN1M2
uaguucuuggugcucuuggcu

SEQ ID NO: 89 - RNA, 23 nt, Artificial sequence
  Antisense sequence for siAN2M2
uaguucuuggugcucuuggcuug

SEQ ID NO: 90 - RNA, 19 nt, Artificial sequence
  Sense sequence for siAN1M3
ccaagagcaccaagaacua

SEQ ID NO: 91 - RNA, 21 nt, Artificial sequence
  Sense sequence for siAN2M3
agccaagagcaccaagaacua

SEQ ID NO: 92 - RNA, 19 nt, Artificial sequence
  Sense sequence for siAN1M1S
ccaagagcaccaagaacua

SEQ ID NO: 93 - RNA, 21 nt, Artificial sequence
  Antisense sequence for siAN1M1S
uaguucuuggugcucuuggcu

SEQ ID NO: 94 - RNA, 21 nt, Artificial sequence
  Sense sequence for siAN2M1S
agccaagagcaccaagaacua

SEQ ID NO: 95 - RNA, 23 nt, Artificial sequence
  Antisense sequence for siAN2M1S
uaguucuuggugcucuuggcuug

SEQ ID NO: 96 - RNA, 21 nt, Artificial sequence
  Antisense sequence for siAN1M2S
uaguucuuggugcucuuggcu

SEQ ID NO: 97 - RNA, 23 nt, Artificial sequence
  Antisense sequence for siAN2M2S
uaguucuuggugcucuuggcuug

SEQ ID NO: 98 - RNA, 19 nt, artificial sequence
  Sense sequence for siAN1M3S
ccaagagcaccaagaacua

SEQ ID NO: 99 - RNA, 21 nt, Artificial sequence
  Sense sequence for siAN2M3S
agccaagagcaccaagaacua

SEQ ID NO: 100 - RNA, 21 nt, Artificial sequence
  Antisense sequence for siAN1M1P1
uaguucuuggugcucuuggcu

SEQ ID NO: 101 - RNA, 23 nt, Artificial sequence
  Antisense sequence for siAN2M1P1
uaguucuuggugcucuuggcuug

SEQ ID NO: 102 - RNA, 21 nt, Artificial sequence
  Antisense sequence for siAN1M2P1
uaguucuuggugcucuuggcu

SEQ ID NO: 103 - RNA, 23 nt, Artificial sequence
  Antisense sequence for siAN2M2P1
uaguucuuggugcucuuggcuug

SEQ ID NO: 104 - RNA, 21 nt, Artificial sequence
  Antisense sequence for siAN1M1SP1
uaguucuuggugcucuuggcu

SEQ ID NO: 105 - RNA, 23 nt, Artificial sequence
  Antisense sequence for siAN2M1SP1
uaguucuuggugcucuuggcuug

SEQ ID NO: 106 - RNA, 21 nt, Artificial sequence
  Antisense sequence for siAN1M3SP1
uaguucuuggugcucuuggcu

SEQ ID NO: 107 - RNA, 23 nt, Artificial sequence
  Antisense sequence for siAN2M3SP1
uaguucuuggugcucuuggcuug

SEQ ID NO: 108 - RNA, 19 nt, Artificial sequence
  Sense sequence for siAP1
caauaaagcuggacaagaa

SEQ ID NO: 109 - RNA, 21 nt, Artificial sequence
  Antisense sequence for siAP1
uucuuguccagcuuuauuggg

SEQ ID NO: 110 - RNA, 21 nt, Artificial sequence
  Sense sequence for siAP2
cccaauaaagcuggacaagaa

SEQ ID NO: 111 - RNA, 23 nt, Artificial sequence
  Antisense sequence for siAP2
uucuuguccagcuuuauugggag

SEQ ID NO: 112 - RNA, 19 nt, Artificial sequence
  Sense sequence for siAP1M1
caauaaagcuggacaagaa

SEQ ID NO: 113 - RNA, 21 nt, artificial sequence
  Antisense sequence for siAP1M1
uucuuguccagcuuuauuggg

SEQ ID NO: 114 - RNA, 21 nt, Artificial sequence
  Sense sequence for siAP2M1
cccaauaaagcuggacaagaa

SEQ ID NO: 115 - RNA, 23 nt, Artificial sequence
  Antisense sequence for siAP2M1
uucuuguccagcuuuauugggag

SEQ ID NO: 116 - RNA, 19 nt, Artificial sequence
  Sense sequence for siAP1M2
caauaaagcuggacaagaa

SEQ ID NO: 117 - RNA, 21 nt, Artificial sequence
  Antisense sequence for siAP1M2
uucuuguccagcuuuauuggg

SEQ ID NO: 118 - RNA, 21 nt, Artificial sequence
  Sense sequence for siAP2M2
cccaauaaagcuggacaagaa

SEQ ID NO: 119 - RNA, 23 nt, Artificial sequence
  Antisense sequence for siAP2M2
uucuuguccagcuuuauugggag

SEQ ID NO: 120 - RNA, 19 nt, Artificial sequence
  Sense sequence for siAP1M1S
caauaaagcuggacaagaa

SEQ ID NO: 121 - RNA, 21 nt, Artificial sequence
  Antisense sequence for siAP1M1S
uucuuguccagcuuuauuggg

SEQ ID NO: 122 - RNA, 21 nt, Artificial sequence
  Sense sequence for siAP2M1S
cccaauaaagcuggacaagaa

SEQ ID NO: 123 - RNA, 23 nt, Artificial sequence
  Antisense sequence for siAP2M1S
uucuuguccagcuuuauugggag

SEQ ID NO: 124 - RNA, 19 nt, Artificial sequence
  Sense sequence for siAP1M2S
caauaaagcuggacaagaa

SEQ ID NO: 125 - RNA, 21 nt, Artificial sequence
  Antisense sequence for siAP1M2S
uucuuguccagcuuuauuggg

SEQ ID NO: 126 - RNA, 21 nt, artificial sequence
  Sense sequence for siAP2M2S
cccaauaaagcuggacaagaa

SEQ ID NO: 127 - RNA, 23 nt, Artificial sequence
  Antisense sequence for siAP2M2S
uucuuguccagcuuuauugggag

SEQ ID NO: 128 - RNA, 21 nt, Artificial sequence
  Antisense sequence for siAP1M1P1
uucuuguccagcuuuauuggg

SEQ ID NO: 129 - RNA, 23 nt, Artificial sequence
  Antisense sequence for siAP2M1P1
uucuuguccagcuuuauugggag

SEQ ID NO: 130 - RNA, 21 nt, Artificial sequence
  Antisense sequence for siAP1M2P1
uucuuguccagcuuuauuggg

SEQ ID NO: 131 - RNA, 23 nt, Artificial sequence
  Antisense sequence for siAP2M2P1
uucuuguccagcuuuauugggag

SEQ ID NO: 132 - RNA, 21 nt, Artificial sequence
  Antisense sequence for siAP1M1SP1
uucuuguccagcuuuauuggg

SEQ ID NO: 133 - RNA, 23 nt, Artificial sequence
  Antisense sequence for siAP2M1SP1
uucuuguccagcuuuauugggag

SEQ ID NO: 134 - RNA, 21 nt, Artificial sequence
  Antisense sequence for siAP1M2SP1
uucuuguccagcuuuauuggg

SEQ ID NO: 135 - RNA, 23 nt, Artificial sequence
  Antisense sequence for siAP2M2SP1
uucuuguccagcuuuauugggag

SEQ ID NO: 136 - RNA, 21 nt, Artificial sequence
  Antisense sequence for L10-siHBa1M1P
uuugaaguaugccucaagguu

SEQ ID NO: 137 - RNA, 21 nt, Artificial sequence
  Antisense sequence for L10-siHBa1M2P
uuugaaguaugccucaagguu

SEQ ID NO: 138 - RNA, 23 nt, Artificial sequence
  Antisense sequence for L10-siHBa2M1P
uuugaaguaugccucaaggucgg

SEQ ID NO: 139 - RNA, 23 nt, Artificial sequence
  Antisense sequence for L10-siHBa2M2P
uuugaaguaugccucaaggucgg

SEQ ID NO: 140 - RNA, 21 nt, Artificial sequence
  Antisense sequence for L10-siHBa1M1SP
uuugaaguaugccucaagguu

SEQ ID NO: 141 - RNA, 21 nt, Artificial sequence
  Antisense sequence for L10-siHBa1M2SP
uuugaaguaugccucaagguu

SEQ ID NO: 142 - RNA, 23 nt, Artificial sequence
  Antisense sequence for L10-siHBa2M1SP
uuugaaguaugccucaaggucgg

SEQ ID NO: 143 - RNA, 23 nt, Artificial sequence
  Antisense sequence for L10-siHBa2M2SP
uuugaaguaugccucaaggucgg

SEQ ID NO: 144 - RNA, 19 nt, Artificial sequence
  Sense sequence for L10-siHBa1M3SP
ccuugaggcauacuucaaa

SEQ ID NO: 145 - RNA, 21 nt, Artificial sequence
  Antisense sequence for L10-siHBa1M4SP
uuugaaguaugccucaagguu

SEQ ID NO: 146 - RNA, 21 nt, Artificial sequence
  Antisense sequence for L10-siHBb1M1SP
uagaagaugaggcauagcagc

SEQ ID NO: 147 - RNA, 21 nt, Artificial sequence
  Antisense sequence for L10-siHBb2M1SP
uagaagaugaggcauagcauu

SEQ ID NO: 148 - RNA, 21 nt, Artificial sequence
  Antisense sequence for L10-siHBb1M2SP
uagaagaugaggcauagcagc

SEQ ID NO: 149 - RNA, 21 nt, Artificial sequence
  Antisense sequence for L10-siHBb2M2SP
uagaagaugaggcauagcauu

SEQ ID NO: 150 - RNA, 21 nt, Artificial sequence
  Sense sequence for L10-siHBb1M3SP
uagaagaugaggcauagcagc

SEQ ID NO: 151 - RNA, 21 nt, Artificial sequence
  Antisense sequence for L10-siHBb1M4SP
uagaagaugaggcauagcagc

SEQ ID NO: 152 - RNA, 21 nt, Artificial sequence
  Sense sequence for L10-siHBb4M1SP
gcugcuaugccucaucuucua

SEQ ID NO: 153 - RNA, 23 nt, Artificial sequence
  Antisense sequence for L10-siHBb4M1SP
uagaagaugaggcauagcagcgc

SEQ ID NO: 154 - RNA, 21 nt, Artificial sequence
  Antisense sequence for L10-siHBc1M1SP
ucagaugagaaggcacagacg

SEQ ID NO: 155 - RNA, 21 nt, Artificial sequence
  Antisense sequence for L10-siHBc1M2SP
ucagaugagaaggcacagacg

SEQ ID NO: 156 - RNA, 19 nt, Artificial sequence
  Sense sequence for L10-siHBc1M3SP
ucugugccuucucaucuga

SEQ ID NO: 157 - RNA, 21 nt, Artificial sequence
  Antisense sequence for L10-siHBc1M4SP
ucagaugagaaggcacagacg

SEQ ID NO: 158 - RNA, 21 nt, Artificial sequence
  Sense sequence for L10-siHBc2M1SP
cgucugugccuucucaucuga

SEQ ID NO: 159 - RNA, 23 nt, Artificial sequence
  Antisense sequence for L10-siHBc2M1SP
ucagaugagaaggcacagacggg

SEQ ID NO: 160 - RNA, 21 nt, Artificial sequence
  Antisense sequence for L10-siHBd1M1SP
uugaagcgaagugcacacggu

SEQ ID NO: 161 - RNA, 21 nt, Artificial sequence
  Antisense sequence for L10-siHBd1M2SP
uugaagcgaagugcacacggu

SEQ ID NO: 162 - RNA, 19 nt, Artificial sequence
  Sense sequence for L10-siHBd1M3SP
cgugugcacuucgcuucaa

SEQ ID NO: 163 - RNA, 21 nt, Artificial sequence
  Antisense sequence for L10-siHBd1M4SP
ucagaugagaaggcacagacg

SEQ ID NO: 164 - RNA, 21 nt, Artificial sequence
  Sense sequence for L10-siHBd2M1SP
accgugugcacuucgcuucaa

SEQ ID NO: 165 - RNA, 23 nt, Artificial sequence
  Antisense sequence for L10-siHBd2M1SP
uugaagcgaagugcacacggucc

SEQ ID NO: 166 - RNA, 21 nt, Artificial sequence
  Antisense sequence for L10-siAN1M1P
uaguucuuggugcucuuggcu

SEQ ID NO: 167 - RNA, 23 nt, Artificial sequence
  Antisense sequence for L10-siAN2M1P
uaguucuuggugcucuuggcuug

SEQ ID NO: 168 - RNA, 21 nt, Artificial sequence
  Antisense sequence for L10-siAN1M2P
uaguucuuggugcucuuggcu

SEQ ID NO: 169 - RNA, 23 nt, Artificial sequence
  Antisense sequence for L10-siAN2M2P
uaguucuuggugcucuuggcuug

SEQ ID NO: 170 - RNA, 21 nt, Artificial sequence
  Antisense sequence for L10-siAN1M1SP
uaguucuuggugcucuuggcu

SEQ ID NO: 171 - RNA, 23 nt, Artificial sequence
  Antisense sequence for L10-siAN2M1SP
uaguucuuggugcucuuggcuug

SEQ ID NO: 172 - RNA, 21 nt, Artificial sequence
  Antisense sequence for L10-siAN1M2SP
uaguucuuggugcucuuggcu

SEQ ID NO: 173 - RNA, 23 nt, Artificial sequence
  Antisense sequence for L10-siAN2M2SP
uaguucuuggugcucuuggcuug

SEQ ID NO: 174 - RNA, 21 nt, Artificial sequence
  Antisense sequence for L10-siAN1M4S
uaguucuuggugcucuuggcu

SEQ ID NO: 175 - RNA, 21 nt, artificial sequence
  Antisense sequence for L10-siAN1M4SP
uaguucuuggugcucuuggcu

SEQ ID NO: 176 - RNA, 19 nt, Artificial sequence
  Sense sequence for L10-siAN1M5S
ccaagagcaccaagaacua

SEQ ID NO: 177 - RNA, 21 nt, Artificial sequence
  Antisense sequence for L10-siAN1M5S
uaguucuuggugcucuuggcu

SEQ ID NO: 178 - RNA, 21 nt, Artificial sequence
  Antisense sequence for L10-siAN1M5SP
uaguucuuggugcucuuggcu

SEQ ID NO: 179 - RNA, 21 nt, Artificial sequence
  Antisense sequence for L10-siAP1M1P
uucuuguccagcuuuauuggg

SEQ ID NO: 180 - RNA, 23 nt, Artificial sequence
  Antisense sequence for L10-siAP2M1P
uucuuguccagcuuuauugggag

SEQ ID NO: 181 - RNA, 21 nt, Artificial sequence
  Antisense sequence for L10-siAP1M2P
uucuuguccagcuuuauuggg

SEQ ID NO: 182 - RNA, 23 nt, Artificial sequence
  Antisense sequence for L10-siAP2M2P
uucuuguccagcuuuauugggag

SEQ ID NO: 183 - RNA, 21 nt, Artificial sequence
  Antisense sequence for L10-siAP1M1SP
uucuuguccagcuuuauuggg

SEQ ID NO: 184 - RNA, 23 nt, Artificial sequence
  Antisense sequence for L10-siAP2M1SP
uucuuguccagcuuuauugggag

SEQ ID NO: 185 - RNA, 21 nt, Artificial sequence
  Antisense sequence for L10-siAP1M2SP
uucuuguccagcuuuauuggg

SEQ ID NO: 186 - RNA, 23 nt, Artificial sequence
  Antisense sequence for L10-siAP2M2SP
uucuuguccagcuuuauugggag

SEQ ID NO: 187 - DNA, 20 bp, Artificial sequence
  upstream primer for mTTR
ccgtctgtgccttctcatct

SEQ ID NO: 188 - DNA, 20 bp, Artificial sequence
  downstream primer for mTTR
taatctcctcccccaactcc

SEQ ID NO: 189 - DNA, 20 bp, Artificial sequence
  upstream primer for GAPDH
agaaggctggggctcatttg

SEQ ID NO: 190 - DNA, 20 bp, Artificial sequence
  downstream primer for GAPDH
aggggccatccacagtcttc

SEQ ID NO: 191 - DNA, 24 bp, Artificial sequence
  upstream primer for β-actin
agcttctttgcagctccttcgttg

SEQ ID NO: 192 - DNA, 24 bp, Artificial sequence
  downstream primer for β-actin
ttctgacccattcccaccatcaca

SEQ ID NO: 193 - DNA, 21 bp, Artificial sequence
  upstream primer for HBV
cgtttctcctggctcagttta

SEQ ID NO: 194 - DNA, 21 bp, Artificial sequence
  downstream primer for HBV
cagcggtaaaaagggactcaa

SEQ ID NO: 195 - RNA, 21 nt, Artificial sequence
  Sense sequence for AD-65695
acauauuugaucagucuuuuu

SEQ ID NO: 196 - RNA, 23 nt, Artificial sequence
  Antisense sequence for AD-65695
aaaaagacugaucaaauauguug

SEQ ID NO: 197 - RNA, 21 nt, Artificial sequence
  Sense sequence for AD-69535
gcuuaaaagggacaguauuca

SEQ ID NO: 198 - RNA, 23 nt, Artificial sequence
  Antisense sequence for AD-69535
ugaauacugucccuuuuaagcaa

SEQ ID NO: 199 - DNA, 23 bp, Artificial sequence
  upstream primer for mouse ANGPTL3
gaggagcagctaaccaacttaat

SEQ ID NO: 200 - DNA, 23 bp, Artificial sequence
  downstream primer for mouse ANGPTL3
tctgcatgtgctgttgacttaat

SEQ ID NO: 201 - DNA, 24 bp, artificial sequence
  upstream primer for mouse GAPDH
aactttggcattgtggaagggctc

SEQ ID NO: 202 - DNA, 24 bp, Artificial sequence
  downstream primer for mouse GAPDH
tggaagagtgggagttgctgttga

SEQ ID NO: 203 - RNA, 21 nt, Artificial sequence
  Antisense sequence for W8-siAN1M3SPs
uaguucuuggugcucuuggcu

SEQ ID NO: 204 - RNA, 21 nt, Artificial sequence
  Sense sequence for L10-simTTR
aacaguguucuugcucuauaa

SEQ ID NO: 205 - RNA, 23 nt, Artificial sequence
  Antisense sequence for L10-simTTR
uuauagagcaagaacacuguuuu

SEQ ID NO: 206 - RNA, 19 nt, Artificial sequence
  Sense sequence for L10-siHBa1M2Sps
ccuugaggcauacuucaaa

SEQ ID NO: 207 - RNA, 21 nt, Artificial sequence
  Antisense sequence for L10-siHBa1M2Sps
uuugaaguaugccucaagguu

SEQ ID NO: 208 - RNA, 19 nt, Artificial sequence
  Sense sequence for L10- siHBa1M2Sp
ccuugaggcauacuucaaa

SEQ ID NO: 209 - RNA, 21 nt, Artificial sequence
  Antisense sequence for L10- siHBa1M2Sp
uuugaaguaugccucaagguu

SEQ ID NO: 210 - RNA, 19 nt, Artificial sequence
  Sense sequence for L10-siHBa1M1Sp
ccuugaggcauacuucaaa

SEQ ID NO: 211 - RNA, 21 nt, Artificial sequence
  Antisense sequence for L10-siHBa1M1Sp
uuugaaguaugccucaagguu

SEQ ID NO: 212 - RNA, 19 nt, Artificial sequence
  Sense sequence for L10- siHBa1M1SpsT
ccuugaggcauacuucaaa

SEQ ID NO: 213 - RNA, 20 nt, Artificial sequence
  Antisense sequence for L10- siHBa1M1SpsT
uugaaguaugccucaagguu

SEQ ID NO: 214 - RNA, 19 nt, Artificial sequence
  Sense sequence for L10-siHBa1M1Sps
ccuugaggcauacuucaaa

SEQ ID NO: 215 - RNA, 21 nt, Artificial sequence
  Antisense sequence for L10-siHBa1M1Sps
uuugaaguaugccucaagguu

SEQ ID NO: 216 - RNA, 19 nt, Artificial sequence
  Sense sequence for P10-siHBa1M2SP
ccuugaggcauacuucaaa

SEQ ID NO: 217 - RNA, 21 nt, Artificial sequence
  Antisense sequence for P10-siHBa1M2SP
uuugaaguaugccucaagguu

SEQ ID NO: 218 - RNA, 19 nt, Artificial sequence
  Sense sequence for W8-siHBa1M2SP
ccuugaggcauacuucaaa

SEQ ID NO: 219 - RNA, 21 nt, Artificial sequence
  Antisense sequence for W8-siHBa1M2SP
uuugaaguaugccucaagguu

SEQ ID NO: 220 - RNA, 19 nt, Artificial sequence
  Sense sequence for Z5-siHBa1M2SP
ccuugaggcauacuucaaa

SEQ ID NO: 221 - RNA, 21 nt, Artificial sequence
  Antisense sequence for Z5-siHBa1M2SP
uuugaaguaugccucaagguu

SEQ ID NO: 222 - RNA, 19 nt, Artificial sequence
  Sense sequence for L10-siP1M1Sp
gaaaguaugucaacgaaua

SEQ ID NO: 223 - RNA, 21 nt, Artificial sequence
  Antisense sequence for L10-siP1M1Sp
uauucguugacauacuuucuu

SEQ ID NO: 224 - RNA, 19 nt, Artificial sequence
  Sense sequence for L10-siP1M1SP
gaaaguaugucaacgaaua

SEQ ID NO: 225 - RNA, 21 nt, Artificial sequence
  Antisense sequence for L10-siP1M1SP
uauucguugacauacuuucuu

SEQ ID NO: 226 - RNA, 21 nt, Artificial sequence
  Sense sequence for L10-siAN2M1Sp
agccaagagcaccaagaacua

SEQ ID NO: 227 - RNA, 23 nt, Artificial sequence
  Antisense sequence for L10-siAN2M1Sp
uaguucuuggugcucuuggcuug

SEQ ID NO: 228 - RNA, 19 nt, Artificial sequence
  Sense sequence for L10-siAP1M1Sp
caauaaagcuggacaagaa

SEQ ID NO: 229 - RNA, 21 nt, Artificial sequence
  Antisense sequence for L10-siAP1M1Sp
uucuuguccagcuuuauuggg

SEQ ID NO: 230 - RNA, 19 nt, Artificial sequence
  Sense sequence for L10-siAP1M1Sps
caauaaagcuggacaagaa

SEQ ID NO: 231 - RNA, 21 nt, Artificial sequence
  Antisense sequence for L10-siAP1M1Sps
uucuuguccagcuuuauuggg

SEQ ID NO: 232 - RNA, 19 nt, Artificial sequence
  Sense sequence for K4-simTTR
caauaaagcuggacaagaa

SEQ ID NO: 233 - RNA, 21 nt, Artificial sequence
  Antisense sequence for K4-simTTR
uucuuguccagcuuuauuggg

SEQ ID NO: 234 - RNA, 19 nt, Artificial sequence
  Sense sequence for AD-66810
caauaaagcuggacaagaa

SEQ ID NO: 235 - RNA, 21 nt, Artificial sequence
  Antisense sequence for AD-66810
uucuuguccagcuuuauuggg

SEQ ID NO: 236 - RNA, 21 nt, Artificial sequence
  Sense sequence for X2M2
ccuugaggcauacuucaaatt

SEQ ID NO: 237 - RNA, 21 nt, Artificial sequence
  Antisense sequence for X2M2
uuugaaguaugccucaaggtt

SEQ ID NO: 238 - DNA, 20 bp, Artificial sequence
  upstream primer for HBV
gtcttttgggttttgctgcc

SEQ ID NO: 239 - DNA, 20 bp, Artificial sequence
  downstream primer for HBV
gcaacggggtaaaggttcag

SEQ ID NO: 240 - DNA, 19 bp, Artificial sequence
  upstream primer for β-actin
ggtcggagtcaacggattt

SEQ ID NO: 241 - DNA, 19 bp, Artificial sequence
  downstream primer for β-actin
ccagcatcgccccacttga

SEQ ID NO: 242 - DNA, 20 bp, Artificial sequence
  upstream primer for monkey ANGPTL3
ctggtggtggcatgatgagt

SEQ ID NO: 243 - DNA, 21 bp, Artificial sequence
  downstream primer for monkey ANGPTL3
ctcttctccgctctggcttag

SEQ ID NO: 244 - DNA, 20 bp, Artificial sequence
  upstream primer for monkey GAPDH
gggagccaaaagggtcatca

SEQ ID NO: 245 - DNA, 20 bp, Artificial sequence
  downstream primer for monkey GAPDH
cgtggactgtggtcatgagt

SEQ ID NO: 246 - DNA, 24 bp, Artificial sequence
  upstream primer for mouse β-actin
agcttctttgcagctccttcgttg

SEQ ID NO: 247 - DNA, 24 bp, Artificial sequence
  downstream primer for mouse β-actin
ttctgacccattcccaccatcaca

SEQ ID NO: 248 - DNA, 20 bp, Artificial sequence
  upstream primer for human APOC3
gtgaccgatggcttcagttc

SEQ ID NO: 249 - DNA, 20 bp, Artificial sequence
  downstream primer for human APOC3
atggataggcaggtggactt

SEQ ID NO: 250 - RNA, 19 nt, Artificial sequence
  Sense sequence for comparative sequence 1
ccuugaggcauacuucaaa

SEQ ID NO: 251 - RNA, 21 nt, Artificial sequence
  Antisense sequence for comparative sequence 1
uuugaaguaugccucaagguu